European Patent Application EP 4 589 017 A2, published July 23, 2025. Title: RNA TEMPLATED LIGATION. Applicant: 10X Genomics, Inc. Application EP, filed October 5, 2018. The sequence listing filed with the application follows.

SEQUENCE LISTING (281 sequences)

SEQ ID NO: 1 - RNA, 41 nt, Homo sapiens
  source 1..41: mol_type = unassigned RNA
aacttgtggtagttggagctggtggcgtaggcaagagtgcc

SEQ ID NO: 2 - DNA, 70 bp, synthetic construct
  misc_feature 1..70: note = KRASwt_PLP
  misc_feature 1: note = 5' Phosphate
  source 1..70: mol_type = other DNA
agctccaactaccacaaaaaaaaaaagtagccgtgactatcgactaaaaaaaaaacttgcctacgccacc

SEQ ID NO: 3 - RNA, 22 nt, Homo sapiens
  source 1..22: mol_type = unassigned RNA
tgaggtaggaggttgtatagtt

SEQ ID NO: 4 - RNA, 22 nt, Homo sapiens
  source 1..22: mol_type = unassigned RNA
agaggtagtaggttgcatagtt

SEQ ID NO: 5 - DNA, 65 bp, synthetic construct
  misc_feature 1..65: note = let7-a_PLP_1
  misc_feature 1: note = 5' Phosphate
  source 1..65: mol_type = other DNA
ctactacctcaaaaaaaaaaacctcaatgcacatgtttggctccaaaaaaaaaaaactatacaac

SEQ ID NO: 6 - DNA, 65 bp, synthetic construct
  misc_feature 1..65: note = let7-f_PLP_1
  misc_feature 1: note = 5' Phosphate
  source 1..65: mol_type = other DNA
ctactacctcaaaaaaaaaaacctcaatgcacatgtttggctccaaaaaaaaaaaactatacaat

SEQ ID NO: 7 - DNA, 65 bp, synthetic construct
  misc_feature 1..65: note = let7-e_PLP_1
  misc_feature 1: note = 5' Phosphate
  source 1..65: mol_type = other DNA
ctcctacctcaaaaaaaaaaacctcaatgcacatgtttggctccaaaaaaaaaaaactatacaac

SEQ ID NO: 8 - DNA, 65 bp, synthetic construct
  misc_feature 1..65: note = let7-d_PLP_1
  misc_feature 1: note = 5' Phosphate
  source 1..65: mol_type = other DNA
ctactacctctaaaaaaaaaacctcaatgcacatgtttggctccaaaaaaaaaaaactatgcaac

SEQ ID NO: 9 - DNA, 65 bp, synthetic construct; identical to SEQ ID NO: 5
  misc_feature 1..65: note = let7-a_PLP_RNA_1
  misc_feature 1: note = 5' Phosphate
  misc_feature 65: note = RNA
  source 1..65: mol_type = other DNA

SEQ ID NO: 10 - DNA, 65 bp, synthetic construct; identical to SEQ ID NO: 6
  misc_feature 1..65: note = let7-f_PLP_RNA_1
  misc_feature 1: note = 5' Phosphate
  misc_feature 65: note = RNA
  source 1..65: mol_type = other DNA

SEQ ID NO: 11 - DNA, 65 bp, synthetic construct; identical to SEQ ID NO: 7
  misc_feature 1..65: note = let7-e_PLP_RNA_1
  misc_feature 1: note = 5' Phosphate
  misc_feature 65: note = RNA
  source 1..65: mol_type = other DNA

SEQ ID NO: 12 - DNA, 65 bp, synthetic construct; identical to SEQ ID NO: 8
  misc_feature 1..65: note = let7-d_PLP_RNA_1
  misc_feature 1: note = 5' Phosphate
  misc_feature 65: note = RNA
  source 1..65: mol_type = other DNA

SEQ ID NO: 13 - RNA, 25 nt, synthetic construct
  misc_feature 1..25: note = benchm_templ_C
  source 1..25: mol_type = other RNA
tctcgctgtcatccctatatcctcg

SEQ ID NO: 14 - RNA, 25 nt, synthetic construct
  misc_feature 1..25: note = benchm_templ_A
  source 1..25: mol_type = other RNA
tctcgctgtcatacctatatcctcg

SEQ ID NO: 15 - RNA, 25 nt, synthetic construct
  misc_feature 1..25: note = benchm_templ_G
  source 1..25: mol_type = other RNA
tctcgctgtcatgcctatatcctcg

SEQ ID NO: 16 - RNA, 25 nt, synthetic construct
  misc_feature 1..25: note = benchm_templ_U
  source 1..25: mol_type = other RNA
tctcgctgtcattcctatatcctcg

SEQ ID NO: 17 - DNA, 65 bp, synthetic construct
  misc_feature 1..65: note = 3'T_PLP_2
  misc_feature 1: note = 5' Phosphate
  source 1..65: mol_type = other DNA
atgacagcgagaaaaaaaaaaaagtagccgtgactatcgactaaaaaaaaaacgaggatataggt

SEQ ID NO: 18 - DNA, 65 bp, synthetic construct
  misc_feature 1..65: note = 3'G_PLP_2
  misc_feature 1: note = 5' Phosphate
  source 1..65: mol_type = other DNA
atgacagcgagaaaaaaaaaaaagtagccgtgactatcgactaaaaaaaaaacgaggatataggg

SEQ ID NO: 19 - DNA, 65 bp, synthetic construct
  misc_feature 1..65: note = 3'A_PLP_2
  misc_feature 1: note = 5' Phosphate
  source 1..65: mol_type = other DNA
atgacagcgagaaaaaaaaaaaagtagccgtgactatcgactaaaaaaaaaacgaggatatagga

SEQ ID NO: 20 - DNA, 65 bp, synthetic construct
  misc_feature 1..65: note = 3'C_PLP_2
  misc_feature 1: note = 5' Phosphate
  source 1..65: mol_type = other DNA
atgacagcgagaaaaaaaaaaaagtagccgtgactatcgactaaaaaaaaaacgaggatataggc

SEQ ID NO: 21 - DNA, 65 bp, synthetic construct; identical to SEQ ID NO: 17
  misc_feature 1..65: note = 3'rT_PLP_2
  misc_feature 1: note = 5' Phosphate
  misc_feature 65: note = RNA
  source 1..65: mol_type = other DNA

SEQ ID NO: 22 - DNA, 65 bp, synthetic construct; identical to SEQ ID NO: 18
  misc_feature 1..65: note = 3'rG_PLP_2
  misc_feature 1: note = 5' Phosphate
  misc_feature 65: note = RNA
  source 1..65: mol_type = other DNA

SEQ ID NO: 23 - DNA, 65 bp, synthetic construct; identical to SEQ ID NO: 19
  misc_feature 1..65: note = 3'rA_PLP_2
  misc_feature 1: note = 5' Phosphate
  misc_feature 65: note = RNA
  source 1..65: mol_type = other DNA

SEQ ID NO: 24 - DNA, 65 bp, synthetic construct; identical to SEQ ID NO: 20
  misc_feature 1..65: note = 3'rC_PLP_2
  misc_feature 1: note = 5' Phosphate
  misc_feature 65: note = RNA
  source 1..65: mol_type = other DNA

SEQ ID NO: 25 - DNA, 24 bp, synthetic construct
  misc_feature 1..24: note = Decorator probe_1
  misc_feature 1: note = 5' Phosphate
  misc_feature 21..24: note = 2' O-Me RNA
  source 1..24: mol_type = other DNA
cctcaatgcacatgtttggctcca

SEQ ID NO: 26 - DNA, 21 bp, synthetic construct
  misc_feature 1..21: note = Decorator probe2_2
  misc_feature 1: note = 5' Phosphate
  misc_feature 18..21: note = 2' O-Me RNA
  source 1..21: mol_type = other DNA
agtagccgtgactatcgacta

SEQ ID NO: 27 - RNA, 22 nt, Homo sapiens
  source 1..22: mol_type = unassigned RNA
tgaggtagtaggttgtatagtt

SEQ ID NO: 28 - DNA, 59 bp, synthetic construct
  misc_feature 1..59: note = let-7a_PLP
  source 1..59: mol_type = other DNA
ctactacctcaaaaaaaacctcaatgcacatgtttggctccaaaaaaaaactatacaac

SEQ ID NO: 29 - DNA, 79 bp, synthetic construct
  misc_feature 1..79: note = iLock_1
  source 1..79: mol_type = other DNA
cgcgtgtcgttgccctactacctcaaaaaaaaaaacctcaatgcacatgtttggctccaaaaaaaaaaaactatacaac

SEQ ID NO: 30 - DNA, 79 bp, synthetic construct; identical to SEQ ID NO: 29
  misc_feature 1..79: note = iLock-3_1
  misc_feature 79: note = RNA
  source 1..79: mol_type = other DNA

SEQ ID NO: 31 - DNA, 79 bp, synthetic construct; identical to SEQ ID NO: 29
  misc_feature 1..79: note = iLock-3D_1
  misc_feature 79: note = RNA
  source 1..79: mol_type = other DNA

SEQ ID NO: 32 - DNA, 79 bp, synthetic construct; identical to SEQ ID NO: 29
  misc_feature 1..79: note = iLock-3D5_1
  misc_feature 79: note = RNA
  source 1..79: mol_type = other DNA

SEQ ID NO: 33 - DNA, 79 bp, synthetic construct; identical to SEQ ID NO: 29
  misc_feature 1..79: note = iLock-3DF_1
  misc_feature 1..14: note = RNA
  misc_feature 79: note = RNA
  source 1..79: mol_type = other DNA

SEQ ID NO: 34 - DNA, 79 bp, synthetic construct; identical to SEQ ID NO: 29
  misc_feature 1..79: note = iLock-DF_1
  misc_feature 1..14: note = RNA
  source 1..79: mol_type = other DNA

SEQ ID NO: 35 - RNA, 25 nt, synthetic construct
  misc_feature 1..25: note = benchm_templ_C
  source 1..25: mol_type = other RNA
tctcgctgtcatccctatatcctcg

SEQ ID NO: 36 - RNA, 25 nt, synthetic construct
  misc_feature 1..25: note = benchm_templ_A
  source 1..25: mol_type = other RNA
tctcgctgtcatacctatatcctcg

SEQ ID NO: 37 - RNA, 25 nt, synthetic construct
  misc_feature 1..25: note = benchm_templ_G
  source 1..25: mol_type = other RNA
tctcgctgtcatgcctatatcctcg

SEQ ID NO: 38 - RNA, 25 nt, synthetic construct
  misc_feature 1..25: note = benchm_templ_U
  source 1..25: mol_type = other RNA
tctcgctgtcattcctatatcctcg

SEQ ID NO: 39 - DNA, 79 bp, synthetic construct
  misc_feature 1..79: note = 3'T_iLock_3
  source 1..79: mol_type = other DNA
tatatccctatattatgacagcgagaaaaaaaaaaaagtagccgtgactatcgactaaaaaaaaaacgaggatataggt

SEQ ID NO: 40 - DNA, 79 bp, synthetic construct
  misc_feature 1..79: note = 3'G_iLock_3
  source 1..79: mol_type = other DNA
tatatccctatatgatgacagcgagaaaaaaaaaaaagtagccgtgactatcgactaaaaaaaaaacgaggatataggg

SEQ ID NO: 41 - DNA, 79 bp, synthetic construct
  misc_feature 1..79: note = 3'A_iLock_3
  source 1..79: mol_type = other DNA
tatatccctatataatgacagcgagaaaaaaaaaaaagtagccgtgactatcgactaaaaaaaaaacgaggatatagga

SEQ ID NO: 42 - DNA, 79 bp, synthetic construct
  misc_feature 1..79: note = 3'C_iLock_3
  source 1..79: mol_type = other DNA
tatatccctatatcatgacagcgagaaaaaaaaaaaagtagccgtgactatcgactaaaaaaaaaacgaggatataggc

SEQ ID NO: 43 - DNA, 79 bp, synthetic construct; identical to SEQ ID NO: 39
  misc_feature 1..79: note = 3'U_iLock_RNA_3
  misc_feature 13: note = RNA
  misc_feature 79: note = RNA
  source 1..79: mol_type = other DNA

SEQ ID NO: 44 - DNA, 79 bp, synthetic construct; identical to SEQ ID NO: 40
  misc_feature 1..79: note = 3'G_iLock_RNA_3
  misc_feature 13: note = RNA
  misc_feature 79: note = RNA
  source 1..79: mol_type = other DNA

SEQ ID NO: 45 - DNA, 79 bp, synthetic construct; identical to SEQ ID NO: 41
  misc_feature 1..79: note = 3'A_iLock _RNA_3
  misc_feature 13: note = RNA
  misc_feature 79: note = RNA
  source 1..79: mol_type = other DNA

SEQ ID NO: 46 - DNA, 79 bp, synthetic construct; identical to SEQ ID NO: 42
  misc_feature 1..79: note = 3'C_iLock _RNA_3
  misc_feature 13
  misc_feature 79
  source 1..79: mol_type = other DNA

SEQ ID NO: 47 - DNA, 24 bp, synthetic construct
  misc_feature 1..24: note = Decorator probe_1
  source 1..24: mol_type = other DNA
cctcaatgcacatgtttggctcca

SEQ ID NO: 48 - DNA, 21 bp, synthetic construct
  misc_feature 1..21: note = Decorator probe_2
  source 1..21: mol_type = other DNA
tgcgtctatttagtggagcca

SEQ ID NO: 49 - DNA, 21 bp, synthetic construct
  misc_feature 1..21: note = Decorator probe_3
  source 1..21: mol_type = other DNA
agtagccgtgactatcgacta

SEQ ID NO: 50 - RNA, 22 nt, Homo sapiens
  source 1..22: mol_type = unassigned RNA
tgaggtagtaggttgtatagtt

SEQ ID NO: 51 - RNA, 22 nt, Homo sapiens
  source 1..22: mol_type = unassigned RNA
tgaggtagtagattgtatagtt

SEQ ID NO: 52 - RNA, 22 nt, Homo sapiens
  source 1..22: mol_type = unassigned RNA
tgaggtaggaggttgtatagtt

SEQ ID NO: 53 - RNA, 22 nt, Homo sapiens
  source 1..22: mol_type = unassigned RNA
agaggtagtaggttgcatagtt

SEQ ID NO: 54 - DNA, 69 bp, synthetic construct
  misc_feature 1..69: note = let-7a_seqRNA
  misc_feature 14: note = RNA
  misc_feature 69: note = RNA
  source 1..69: mol_type = other DNA
aaagatgcgatacactacctcatgcgtctatttagtggagcccgctatcttctttaactatacaaccta

SEQ ID NO: 55 - DNA, 69 bp, synthetic construct
  misc_feature 1..69: note = let-7e_seqRNA
  misc_feature 14: note = RNA
  misc_feature 69: note = RNA
  source 1..69: mol_type = other DNA
aaaatgtcgttgccctcctacctcatgcgtctatttagtggagccgcctatcttctttaactatacaac

SEQ ID NO: 56 - DNA, 69 bp, synthetic construct
  misc_feature 1..69: note = let-7d_seqRNA
  misc_feature 14: note = RNA
  misc_feature 69: note = RNA
  source 1..69: mol_type = other DNA
aaaatgtcgttgccctactacctcttgcgtctatttagtggagccatctatcttctttaactatgcaac

SEQ ID NO: 57 - DNA, 69 bp, synthetic construct
  misc_feature 1..69: note = let-7f_seqRNA
  misc_feature 14: note = RNA
  misc_feature 69: note = RNA
  source 1..69: mol_type = other DNA
aaaatgtcgttgctctactacctcatgcgtctatttagtggagcctactatcttctttaactatacaat

SEQ ID NO: 58 - DNA, 69 bp, synthetic construct; identical to SEQ ID NO: 54
  misc_feature 1..69: note = let-7a_seq
  source 1..69: mol_type = other DNA

SEQ ID NO: 59 - DNA, 69 bp, synthetic construct; identical to SEQ ID NO: 55
  misc_feature 1..69: note = let-7e_seq
  source 1..69: mol_type = other DNA

SEQ ID NO: 60 - DNA, 69 bp, synthetic construct; identical to SEQ ID NO: 56
  misc_feature 1..69: note = let-7d_seq
  source 1..69: mol_type = other DNA

SEQ ID NO: 61 - DNA, 69 bp, synthetic construct; identical to SEQ ID NO: 57
  misc_feature 1..69: note = let-7f_seq
  source 1..69: mol_type = other DNA

SEQ ID NO: 62 - DNA, 21 bp, synthetic construct
  misc_feature 1..21: note = Decorator probe
  misc_feature 1: note = 5' Cy3
  source 1..21: mol_type = other DNA
tgcgtctatttagtggagcca

SEQ ID NO: 63 - DNA, 21 bp, synthetic construct
  misc_feature 1..21: note = anchor primer
  misc_feature 1: note = 5' AlexaFluor750
  source 1..21: mol_type = other DNA
tgcgtctatttagtggagcca

SEQ ID NO: 64-67 - skipped (4 entries)

SEQ ID NO: 68 - DNA, 54 bp, Mus musculus
  source 1..54: mol_type = unassigned DNA
ggcctgtacactgacttgagaccaataaaagtgcacaccttaccttacacaaac

SEQ ID NO: 69 - DNA, 94 bp, Homo sapiens
  source 1..94: mol_type = unassigned DNA
tacctgtacactgacttgagaccagttgaataaaagtgcacaccttaaaaatgaaaaaaaaaaaaaaaaaaaaaaaaaaaaaaaaaaaaaaaaa

SEQ ID NO: 70 - DNA, 69 bp, synthetic construct
  misc_feature 1..69: note = Mouse PLP
  source 1..69: mol_type = other DNA
taaggtgtgcaaaaagtagccgtgactatcgactaaaagtagccgtgactatcgactgtttgtgtaagg

SEQ ID NO: 71 - DNA, 68 bp, synthetic construct
  misc_feature 1..68: note = Human PLP
  source 1..68: mol_type = other DNA
taaggtgtgcaagtcggaagtactactctctaaaagtcggaagtactactctctttttttttcatttt

SEQ ID NO: 72 - DNA, 69 bp, synthetic construct; identical to SEQ ID NO: 70
  misc_feature 1..69: note = Mouse cPLP
  misc_feature 69: note = RNA
  source 1..69: mol_type = other DNA

SEQ ID NO: 73 - DNA, 68 bp, synthetic construct; identical to SEQ ID NO: 71
  misc_feature 1..68: note = Human cPLP
  misc_feature 68: note = RNA
  source 1..68: mol_type = other DNA

SEQ ID NO: 74 - DNA, 83 bp, synthetic construct
  misc_feature 1..83: note = Mouse iLock
  source 1..83: mol_type = other DNA
tatatccctatatgtaaggtgtgcaaaaagtagccgtgactatcgactaaaagtagccgtgactatcgactgtttgtgtaagg

SEQ ID NO: 75 - DNA, 82 bp, synthetic construct
  misc_feature 1..82: note = Human iLock
  source 1..82: mol_type = other DNA
tatatccctatatttaaggtgtgcaagtcggaagtactactctctaaaagtcggaagtactactctctttttttttcatttt

SEQ ID NO: 76 - DNA, 83 bp, synthetic construct; identical to SEQ ID NO: 74
  misc_feature 1..83: note = Mouse ciLock
  misc_feature 14: note = RNA
  misc_feature 83: note = RNA
  source 1..83: mol_type = other DNA

SEQ ID NO: 77 - DNA, 82 bp, synthetic construct; identical to SEQ ID NO: 75
  misc_feature 1..82: note = Human ciLock
  misc_feature 14: note = RNA
  misc_feature 82: note = RNA
  source 1..82: mol_type = other DNA

SEQ ID NO: 78 - RNA, 37 nt, synthetic construct
  misc_feature 1..37: note = miR21_BIO
  source 1..37: mol_type = other RNA
ttttttttttttttttagcttatcagactgatgttga

SEQ ID NO: 79 - DNA, 55 bp, synthetic construct
  misc_feature 1..55: note = >miR21B2DO_PLP
  misc_feature 1: note = 5' Phosphate
  source 1..55: mol_type = other DNA
ctgataagctagccgaatctaagagtagccgtgactatcgactaaaactacacca

SEQ ID NO: 80 - DNA, 68 bp, synthetic construct
  misc_feature 1..68: note = >miR21B2DO_iLock
  source 1..68: mol_type = other DNA
ccgtcgctgcgttctgataagctaaaaaaaagtagccgtgactatcgactaaaaaaatcaacatcagt

SEQ ID NO: 81 - DNA, 66 bp, synthetic construct
  misc_feature 1..66: note = > miR21 B2DO_rPLP
  misc_feature 1: note = 5' Phosphate
  misc_feature 1: note = Phosphate
  misc_feature 66: note = RNA
  source 1..66: mol_type = other DNA
ctgataagctagccgaatctaagagtagccgtgactatcgactaaaactacaccatcaacatcagt

SEQ ID NO: 82 - DNA, 68 bp, synthetic construct; identical to SEQ ID NO: 80
  misc_feature 1..68: note = >miR21B2DO_RiLock
  misc_feature 13: note = RNA
  misc_feature 68: note = RNA
  source 1..68: mol_type = other DNA

SEQ ID NO: 83 - DNA, 20 bp, synthetic construct
  misc_feature 1..20: note = >B2DO_Cy3
  misc_feature 1: note = 5' Cy3
  source 1..20: mol_type = other DNA
agtagccgtgactatcgact

SEQ ID NO: 84 - DNA, 22 bp, synthetic construct
  misc_feature 1..22: note = >antimiR21_FAM
  misc_feature 1: note = 5' FAM
  source 1..22: mol_type = other DNA
tcaacatcagtctgataagcta

SEQ ID NO: 85 - DNA, 99 bp, Homo sapiens
  source 1..99: mol_type = unassigned DNA
acattttcattatttttattataaggcctgctgaaaatgactgaatataaacttgtggtagttggagctggtggcgtaggcaagagtgccttgacgata

SEQ ID NO: 86 - DNA, 77 bp, synthetic construct
  misc_feature 1..77: note = wt KRAS PLP
  source 1..77: mol_type = other DNA
agctccaactaccacaaagtcgatagtcacggctactcagacgtaacgcgttcagtgatgcccttgcctacgccacc

SEQ ID NO: 87 - RNA, 41 nt, Homo sapiens; identical to SEQ ID NO: 1
  source 1..41: mol_type = unassigned RNA

SEQ ID NO: 88 - DNA, 77 bp, synthetic construct; identical to SEQ ID NO: 86
  misc_feature 1..77: note = chim wt KRAS PLP
  misc_feature 77: note = RNA
  source 1..77: mol_type = other DNA

SEQ ID NO: 89 - DNA, 77 bp, synthetic construct; identical to SEQ ID NO: 86
  misc_feature 1..77: note = chim wt KRAS PLP_2
  misc_feature 76..77: note = RNA
  source 1..77: mol_type = other DNA

SEQ ID NO: 90 - DNA, 80 bp, synthetic construct
  misc_feature 1..80: note = mut KRAS PLP
  source 1..80: mol_type = other DNA
agctccaactaccacaacctcaatgcacatgtttggctcccagacgtaacgcgttcagtgatgcccttgcctacgccact

SEQ ID NO: 91 - DNA, 80 bp, synthetic construct; identical to SEQ ID NO: 90
  misc_feature 1..80: note = chim mut KRAS PLP
  misc_feature 80: note = RNA
  source 1..80: mol_type = other DNA

SEQ ID NO: 92 - DNA, 15 bp, synthetic construct
  misc_feature 1..15: note = RCA primer
  source 1..15: mol_type = other DNA
catcactgaacgcgt

SEQ ID NO: 93 - DNA, 23 bp, synthetic construct
  misc_feature 1..23: note = mut DO-Cy5
  source 1..23: mol_type = other DNA
cctcaatgcacatgtttggctcc

SEQ ID NO: 94 - DNA, 20 bp, synthetic construct
  misc_feature 1..20: note = wt DO-Cy3
  source 1..20: mol_type = other DNA
agtcgatagtcacggctact

SEQ ID NO: 95 - DNA, 91 bp, synthetic construct
  misc_feature 1..91: note = KRAS wt invader chim 3-5
  misc_feature 14: note = RNA
  misc_feature 91: note = RNA
  source 1..91: mol_type = other DNA
tatatccctatatcagctccaactaccacaaagtcgatagtcacggctactcagacgtaacgcgttcagtgatgcccttgcctacgccacc

SEQ ID NO: 96 - DNA, 91 bp, synthetic construct; identical to SEQ ID NO: 95
  misc_feature 1..91: note = KRAS wt invader chim 3
  misc_feature 14: note = RNA
  misc_feature 91: note = RNA
  source 1..91: mol_type = other DNA

SEQ ID NO: 97 - DNA, 94 bp, synthetic construct
  misc_feature 1..94: note = KRAS mut invader chim 3-5
  misc_feature 14: note = RNA
  misc_feature 94: note = RNA
  source 1..94: mol_type = other DNA
tatatccctatattagctccaactaccacaacctcaatgcacatgtttggctcccagacgtaacgcgttcagtgatgcccttgcctacgccact

SEQ ID NO: 98 - DNA, 94 bp, synthetic construct; identical to SEQ ID NO: 97
  misc_feature 1..94: note = KRAS mut invader chim 3
  misc_feature 14: note = RNA
  misc_feature 94: note = RNA
  source 1..94: mol_type = other DNA

SEQ ID NO: 99 - DNA, 94 bp, synthetic construct
  misc_feature 1..94: note = KRAS gapfill invader
  source 1..94: mol_type = other DNA
tatatctctatatagctccaactaccacaagtagtcgatagtcacggctactcagacgtaacgcgttcagtgatgagtaggcactcttgcctac

SEQ ID NO: 100 - DNA, 19 bp, synthetic construct
  misc_feature 1..19: note = invader_splint_chim
  misc_feature 19: note = RNA
  source 1..19: mol_type = other DNA
tatatctctatatgccacc

SEQ ID NO: 101 - DNA, 19 bp, synthetic construct
  misc_feature 1..19: note = invader_splint
  source 1..19: mol_type = other DNA
tatatctctatatgccacc

SEQ ID NO: 102-103 - skipped (2 entries)

SEQ ID NO: 104 - DNA, 15 bp, synthetic construct
  misc_feature 1..15: note = RCA primer
  source 1..15: mol_type = other DNA
catcactgaacgcgt

SEQ ID NO: 105 - DNA, 20 bp, synthetic construct
  misc_feature 1..20: note = DO-Cy3
  source 1..20: mol_type = other DNA
agtcgatagtcacggctact

SEQ ID NO: 106 - RNA, 41 nt, Homo sapiens; identical to SEQ ID NO: 1
  source 1..41: mol_type = unassigned RNA

SEQ ID NO: 107 - DNA, 57 bp, synthetic construct
  misc_feature 1..57: note = R_KRAS wt1_1
  misc_feature 20: note = RNA
  source 1..57: mol_type = other DNA
agctccaactaccacaacagacgtaacgcgttcagtgatgcccttgcctacgccacc

SEQ ID NO: 108 - DNA, 57 bp, synthetic construct; identical to SEQ ID NO: 107
  misc_feature 1..57: note = R_KRAS wt1_2
  misc_feature 20..21: note = RNA
  misc_feature 29..30: note = RNA
  source 1..57: mol_type = other DNA

SEQ ID NO: 109 - DNA, 57 bp, synthetic construct; identical to SEQ ID NO: 107
  misc_feature 1..57: note = R_KRAS wt1_3
  misc_feature 20..22: note = RNA
  misc_feature 29..30: note = RNA
  source 1..57: mol_type = other DNA

SEQ ID NO: 110 - DNA, 57 bp, synthetic construct; identical to SEQ ID NO: 107
  misc_feature 1..57: note = R_KRAS wt1_4
  misc_feature 20..23: note = RNA
  misc_feature 29..30: note = RNA
  source 1..57: mol_type = other DNA

SEQ ID NO: 111 - DNA, 57 bp, synthetic construct; identical to SEQ ID NO: 107
  misc_feature 1..57: note = R_KRAS wt1_5
  misc_feature 20..24: note = RNA
  misc_feature 29..30: note = RNA
  source 1..57: mol_type = other DNA

SEQ ID NO: 112 - DNA, 57 bp, synthetic construct; identical to SEQ ID NO: 107
  misc_feature 1..57: note = R_KRAS wt1_7
  misc_feature 20..26: note = RNA
  misc_feature 29..30: note = RNA
  source 1..57: mol_type = other DNA

SEQ ID NO: 113 - DNA, 57 bp, synthetic construct; identical to SEQ ID NO: 107
  misc_feature 1..57: note = R_KRAS wt1_6S
  misc_feature 20..21: note = RNA
  misc_feature 24..25: note = RNA
  misc_feature 28..29: note = RNA
  source 1..57: mol_type = other DNA

SEQ ID NO: 114 - DNA, 50 bp, synthetic construct
  misc_feature 1..50: note = R_KRAS wt1_DNA
  source 1..50: mol_type = other DNA
agctccaactaccacaaaaaaaaaaaaaaaaaaaacttgcctacgccacc

SEQ ID NO: 115 - DNA, 50 bp, synthetic construct; identical to SEQ ID NO: 114
  misc_feature 1..50: note = R_KRAS wt1_RNA
  misc_feature 50: note = RNA
  source 1..50: mol_type = other DNA

SEQ ID NO: 116 - DNA, 22 bp, synthetic construct
  misc_feature 1..22: note = Decorator probe [1]
  misc_feature 19..22: note = 2' O-Me RNA
  source 1..22: mol_type = other DNA
cctcaatgcacatgtttggctc

SEQ ID NO: 117 - DNA, 20 bp, synthetic construct
  misc_feature 1..20: note = Decorator probe2 [2]
  misc_feature 17..20: note = 2' O-Me RNA
  source 1..20: mol_type = other DNA
agtcgatagtcacggctact

SEQ ID NO: 118 - RNA, 41 nt, Homo sapiens; identical to SEQ ID NO: 1
  source 1..41: mol_type = unassigned RNA

SEQ ID NO: 119 - DNA, 77 bp, synthetic construct; identical to SEQ ID NO: 86
  misc_feature 1..77: note = R_KRAS.0
  source 1..77: mol_type = other DNA

SEQ ID NO: 120 - DNA, 77 bp, synthetic construct; identical to SEQ ID NO: 86
  misc_feature 1..77: note = R_KRAS.1G
  misc_feature 40: note = RNA
  source 1..77: mol_type = other DNA

SEQ ID NO: 121 - DNA, 77 bp, synthetic construct
  misc_feature 1..77: note = R_KRAS.1C
  misc_feature 40: note = RNA
  source 1..77: mol_type = other DNA
agctccaactaccacaaagtcgatagtcacggctactcacacgtaacgcgttcagtgatgcccttgcctacgccacc

SEQ ID NO: 122 - DNA, 77 bp, synthetic construct
  misc_feature 1..77: note = R_KRAS.1A
  misc_feature 40: note = RNA
  source 1..77: mol_type = other DNA
agctccaactaccacaaagtcgatagtcacggctactcaaacgtaacgcgttcagtgatgcccttgcctacgccacc

SEQ ID NO: 123 - DNA, 77 bp, synthetic construct
  misc_feature 1..77: note = R_KRAS.1U
  misc_feature 40: note = RNA
  source 1..77: mol_type = other DNA
agctccaactaccacaaagtcgatagtcacggctactcatacgtaacgcgttcagtgatgcccttgcctacgccacc

SEQ ID NO: 124 - DNA, 77 bp, synthetic construct
  misc_feature 1..77: note = R_KRAS.2G
  misc_feature 40..41: note = RNA
  misc_feature 49..50: note = RNA
  source 1..77: mol_type = other DNA
agctccaactaccacaaagtcgatagtcacggctactcaggcgtaacgcgttcagtgatgcccttgcctacgccacc

SEQ ID NO: 125 - DNA, 77 bp, synthetic construct
  misc_feature 1..77: note = R_KRAS.2C
  misc_feature 40..41: note = RNA
  misc_feature 49..50: note = RNA
  source 1..77: mol_type = other DNA
agctccaactaccacaaagtcgatagtcacggctactcacccgtaacgcgttcagtgatgcccttgcctacgccacc

SEQ ID NO: 126 - DNA, 77 bp, synthetic construct; identical to SEQ ID NO: 122
  misc_feature 1..77: note = R_KRAS.2A
  misc_feature 40..41: note = RNA
  misc_feature 49..50: note = RNA
  source 1..77: mol_type = other DNA

SEQ ID NO: 127 - DNA, 77 bp, synthetic construct
  misc_feature 1..77: note = R_KRAS.2U
  misc_feature 40..41: note = RNA
  misc_feature 49..50: note = RNA
  source 1..77: mol_type = other DNA
agctccaactaccacaaagtcgatagtcacggctactcattcgtaacgcgttcagtgatgcccttgcctacgccacc

SEQ ID NO: 128 - DNA, 18 bp, synthetic construct
  misc_feature 1..18: note = AluI KRAS RO
  source 1..18: mol_type = other DNA
cgccaccagctccaacta

SEQ ID NO: 129 - DNA, 53 bp, synthetic construct
  misc_feature 1..53: note = PE1
  source 1..53: mol_type = other DNA
acactctttccctacacgacgctcttccgatctctggtggcgtaggcaagggc

SEQ ID NO: 130 - DNA, 54 bp, synthetic construct
  misc_feature 1..54: note = PE2
  source 1..54: mol_type = other DNA
gtgactggagttcagacgtgtgctcttccgatctctccaactaccacaaagtcg

SEQ ID NO: 131 - DNA, 77 bp, synthetic construct
  misc_feature 1..77: note = R_KRAS.3G
  misc_feature 40..42: note = RNA
  misc_feature 49..50: note = RNA
  source 1..77: mol_type = other DNA
agctccaactaccacaaagtcgatagtcacggctactcagggttaacgcgttcagtgatgcccttgcctacgccacc

SEQ ID NO: 132 - DNA, 77 bp, synthetic construct; identical to SEQ ID NO: 125
  misc_feature 1..77: note = R_KRAS.3C
  misc_feature 40..42: note = RNA
  misc_feature 49..50: note = RNA
  source 1..77: mol_type = other DNA

SEQ ID NO: 133 - DNA, 77 bp, synthetic construct
  misc_feature 1..77: note = R_KRAS.3A
  misc_feature 40..42: note = RNA
  misc_feature 49..50: note = RNA
  source 1..77: mol_type = other DNA
agctccaactaccacaaagtcgatagtcacggctactcaaaagtaacgcgttcagtgatgcccttgcctacgccacc

SEQ ID NO: 134 - DNA, 78 bp, synthetic construct
  misc_feature 1..78: note = R_KRAS.3U
  misc_feature 40..42: note = RNA
  misc_feature 49..50: note = RNA
  source 1..78: mol_type = other DNA
agctccaactaccacaaagtcgatagtcacggctactcatttcgtaacgcgttcagtgatgcccttgcctacgccacc

SEQ ID NO: 135 - DNA, 77 bp, synthetic construct; identical to SEQ ID NO: 86
  misc_feature 1..77: note = R_KRAS.5
  misc_feature 40..44: note = RNA
  source 1..77: mol_type = other DNA

SEQ ID NO: 136 - DNA, 77 bp, synthetic construct; identical to SEQ ID NO: 86
  misc_feature 1..77: note = R_KRAS.6S
  misc_feature 40..41: note = RNA
  misc_feature 44..45: note = RNA
  misc_feature 48..49: note = RNA
  source 1..77: mol_type = other DNA

SEQ ID NO: 137 - DNA, 77 bp, synthetic construct; identical to SEQ ID NO: 86
  misc_feature 1..77: note = R_KRAS.3
  misc_feature 40..42: note = RNA
  misc_feature 48..50: note = RNA
  source 1..77: mol_type = other DNA

SEQ ID NO: 138 - DNA, 77 bp, synthetic construct; identical to SEQ ID NO: 86
  misc_feature 1..77: note = R_KRAS.3S
  misc_feature 40
  misc_feature 42
  misc_feature 44
  source 1..77: mol_type = other DNA

SEQ ID NO: 139 - DNA, 77 bp, synthetic construct; identical to SEQ ID NO: 86
  misc_feature 1..77: note = R_KRAS.2
  misc_feature 40..41: note = RNA
  misc_feature 49..50: note = RNA
  source 1..77: mol_type = other DNA

SEQ ID NO: 140 - DNA, 77 bp, synthetic construct; identical to SEQ ID NO: 86
  misc_feature 1..77: note = R_KRAS.7
  misc_feature 40..46: note = RNA
  source 1..77: mol_type = other DNA

SEQ ID NO: 141 - DNA, 20 bp, synthetic construct
  misc_feature 1..20: note = Detection probe (seq anchor probe)
  misc_feature 1: note = 5' AlexaFluor750
  source 1..20: mol_type = other DNA
tgcgtctatttagtggagcc

SEQ ID NO: 142 - skipped

SEQ ID NO: 143 - DNA, 20 bp, synthetic construct
  misc_feature 1..20: note = Seq library 1st base-G
  misc_feature 20: note = 3' thiophosphate
  source 1..20: mol_type = other DNA
ggctccactaaatagacgca

SEQ ID NO: 144-158 - skipped (15 entries)

SEQ ID NO: 159 - DNA, 95 bp, synthetic construct
  misc_feature 1..95: note = Calb2_1119_RNA
  misc_feature 95: note = RNA
  source 1..95: mol_type = other DNA
catcgcagcggagacgacagctgattcctttgactcacattgcgtctatttagtggagccaatgctatcttctttatacagcgaaggaactcatg

SEQ ID NO: 160 - DNA, 95 bp, synthetic construct
  misc_feature 1..95: note = Calb2_1328_RNA
  misc_feature 95: note = RNA
  source 1..95: mol_type = other DNA
cacacacgtcaagaacacaactgattcctttgactcacattgcgtctatttagtggagccaatgctatcttctttgaagccaaagagaaaaggaa

SEQ ID NO: 161 - DNA, 95 bp, synthetic construct
  misc_feature 1..95: note = Calb2_164_RNA
  misc_feature 95: note = RNA
  source 1..95: mol_type = other DNA
accttcaatgtacccatttcctgattcctttgactcacattgcgtctatttagtggagccaatgctatcttctttaagaagttctctagctcttt

SEQ ID NO: 162 - DNA, 95 bp, synthetic construct
  misc_feature 1..95: note = Calb2_500_RNA
  misc_feature 95: note = RNA
  source 1..95: mol_type = other DNA
aggttcatcatagggcctgtctgattcctttgactcacattgcgtctatttagtggagccaatgctatcttcttttgggtgtactcctggagctt

SEQ ID NO: 163 - DNA, 95 bp, synthetic construct
  misc_feature 1..95: note = Calb2_937_RNA
  misc_feature 95: note = RNA
  source 1..95: mol_type = other DNA
gtcaagagagtcaggacagcctgattcctttgactcacattgcgtctatttagtggagccaatgctatcttctttggggaggtctgggaaggagt

SEQ ID NO: 164 - DNA, 93 bp, synthetic construct
  misc_feature 1..93: note = Calb2_DO3_CCAA_RNA
  misc_feature 93: note = RNA
  source 1..93: mol_type = other DNA
ctcatacagatccttcagctgattcctttgactcacattgcgtctatttagtggagccccaactatcttctttttcatctccttcttgttctt

SEQ ID NO: 165 - DNA, 95 bp, synthetic construct
  misc_feature 1..95: note = Chodl_1164_RNA
  misc_feature 95: note = RNA
  source 1..95: mol_type = other DNA
cgggctagtttttgatcttcctgattcctttgactcacattgcgtctatttagtggagccagtactatcttctttatccacagtgtagactgatt

SEQ ID NO: 166 - DNA, 95 bp, synthetic construct
  misc_feature 1..95: note = Chodl_1798_RNA
  misc_feature 95: note = RNA
  source 1..95: mol_type = other DNA
aaagcaaagaaacagaacaactgattcctttgactcacattgcgtctatttagtggagccagtactatcttcttttcctaaactttatcgaaccc

SEQ ID NO: 167 - DNA, 95 bp, synthetic construct
  misc_feature 1..95: note = Chodl_2071_RNA
  misc_feature 95: note = RNA
  source 1..95: mol_type = other DNA
attctataggcaacatgtgactgattcctttgactcacattgcgtctatttagtggagccagtactatcttctttactctggggagctatttgca

SEQ ID NO: 168 - DNA, 95 bp, synthetic construct
  misc_feature 1..95: note = Chodl_2252_RNA
  misc_feature 95: note = RNA
  source 1..95: mol_type = other DNA
gttctgcttagcatcacactctgattcctttgactcacattgcgtctatttagtggagccagtactatcttctttttaatcattaatatcagtgt

SEQ ID NO: 169 - DNA, 95 bp, synthetic construct
  misc_feature 1..95: note = Chodl_293_RNA
  misc_feature 95: note = RNA
  source 1..95: mol_type = other DNA
tcctactccctccttcccagctgattcctttgactcacattgcgtctatttagtggagccagtactatcttctttttccttgctttcctgctggg

SEQ ID NO: 170 - DNA, 95 bp, synthetic construct
  misc_feature 1..95: note = Chodl_789_RNA
  misc_feature 95: note = RNA
  source 1..95: mol_type = other DNA
gaactgggagctgcttccatctgattcctttgactcacattgcgtctatttagtggagccagtactatcttcttttcatcagtgtaccagtttcg

SEQ ID NO: 171 - DNA, 95 bp, synthetic construct
  misc_feature 1..95: note = Chodl_916_RNA
  misc_feature 95: note = RNA
  source 1..95: mol_type = other DNA
tgttgcacctgtcgtcattcctgattcctttgactcacattgcgtctatttagtggagccagtactatcttctttgcagatgtaattgtgcttca

SEQ ID NO: 172 - DNA, 95 bp, synthetic construct
  misc_feature 1..95: note = Cort_326_RNA
  misc_feature 95: note = RNA
  source 1..95: mol_type = other DNA
cccgggggtaccccctccgacgtgcttgtggtagcaaatatgcgtctatttagtggagcctgatctatcttctttctttcctggctcttggacag

SEQ ID NO: 173 - DNA, 95 bp, synthetic construct
  misc_feature 1..95: note = Cort_529_RNA
  misc_feature 95: note = RNA
  source 1..95: mol_type = other DNA
caaagctgacataagaagaacgtgcttgtggtagcaaatatgcgtctatttagtggagcctgatctatcttctttttctcacagggcaggggagg

SEQ ID NO: 174 - DNA, 95 bp, synthetic construct
  misc_feature 1..95: note = Htr3a_1014_GGAC_RNA
  misc_feature 95: note = RNA
  source 1..95: mol_type = other DNA
agtgtgtctgacacgatgatcgtgcttgtggtagcaaatatgcgtctatttagtggagccggacctatcttcttttaccgatggccgttgctggc

SEQ ID NO: 175 - DNA, 95 bp, synthetic construct
  misc_feature 1..95: note = Htr3a_1309_GTAA_RNA
  misc_feature 95: note = RNA
  source 1..95: mol_type = other DNA
atggctgcagtggtttcccacgtgcttgtggtagcaaatatgcgtctatttagtggagccgtaactatcttctttaagtcctgaggtcctccaac

SEQ ID NO: 176 - DNA, 95 bp, synthetic construct
  misc_feature 1..95: note = Htr3a_1573_TAAC_RNA
  misc_feature 95: note = RNA
  source 1..95: mol_type = other DNA
ccaaatggaccagagagtgacgtgcttgtggtagcaaatatgcgtctatttagtggagcctaacctatcttctttgtgcccactcaagaataatg

SEQ ID NO: 177 - DNA, 95 bp, synthetic construct
  misc_feature 1..95: note = Htr3a_1750_TATT_RNA
  misc_feature 95: note = RNA
  source 1..95: mol_type = other DNA
aagtcagagagacagactggcgtgcttgtggtagcaaatatgcgtctatttagtggagcctattctatcttctttgctttaaagccatgataggg

SEQ ID NO: 178 - DNA, 95 bp, synthetic construct
  misc_feature 1..95: note = Htr3a_1927_TCGC_RNA
  misc_feature 95: note = RNA
  source 1..95: mol_type = other DNA
gcaagacaatttgcttttctcgtgcttgtggtagcaaatatgcgtctatttagtggagcctcgcctatcttctttcagaagtctcaggcatctat

SEQ ID NO: 179 - DNA, 95 bp, synthetic construct
  misc_feature 1..95: note = Htr3a_2045_TGGA_RNA
  misc_feature 95: note = RNA
  source 1..95: mol_type = other DNA
attatcccctgctcccattgcgtgcttgtggtagcaaatatgcgtctatttagtggagcctggactatcttctttttaagatatcatagcatttt

SEQ ID NO: 180 - DNA, 95 bp, synthetic construct
  misc_feature 1..95: note = Htr3a_21_AAGT_RNA
  misc_feature 95: note = RNA
  source 1..95: mol_type = other DNA
gtcccaggcagactgcttttcgtgcttgtggtagcaaatatgcgtctatttagtggagccaagtctatcttctttccacccgctgccaacctcat

SEQ ID NO: 181 - DNA, 95 bp, synthetic construct
  misc_feature 1..95: note = Htr3a_247_CAGC_RNA
  misc_feature 95: note = RNA
  source 1..95: mol_type = other DNA
gtctgacagccttagtagagcgtgcttgtggtagcaaatatgcgtctatttagtggagcccagcctatcttctttttgtagttagccaggaggtg

SEQ ID NO: 182 - DNA, 95 bp, synthetic construct
  misc_feature 1..95: note = Htr3a_424_CGGT_RNA
  misc_feature 95: note = RNA
  source 1..95: mol_type = other DNA
agtccactgcagaaactcatcgtgcttgtggtagcaaatatgcgtctatttagtggagcccggtctatcttctttacattgtcgaagtcctcagg

SEQ ID NO: 183 - DNA, 95 bp, synthetic construct
  misc_feature 1..95: note = Htr3a_89_CACT_RNA
  misc_feature 95: note = RNA
  source 1..95: mol_type = other DNA
ctcagagcagccactcaggacgtgcttgtggtagcaaatatgcgtctatttagtggagcccactctatcttctttcttcccagatgtgggagggc

SEQ ID NO: 184 - DNA, 95 bp, synthetic construct
  misc_feature 1..95: note = Htr3a_955_GCTC_RNA
  misc_feature 95: note = RNA
  source 1..95: mol_type = other DNA
agagactctctcaccgctgtcgtgcttgtggtagcaaatatgcgtctatttagtggagccgctcctatcttctttagaaggagtgtgatcttgaa

SEQ ID NO: 185 - DNA, 95 bp, synthetic construct
  misc_feature 1..95: note = Neurod6_1033_RNA
  misc_feature 95: note = RNA
  source 1..95: mol_type = other DNA
tagaaggattcatatgcactctgattcctttgactcacattgcgtctatttagtggagccttgcctatcttctttactcaggggaggtactttca

SEQ ID NO: 186 - DNA, 95 bp, synthetic construct
  misc_feature 1..95: note = Neurod6_108_RNA
  misc_feature 95: note = RNA
  source 1..95: mol_type = other DNA
ctgctagtgacgtcacagggctgattcctttgactcacattgcgtctatttagtggagccttgcctatcttctttagagctggtacccatgccat

SEQ ID NO: 187 - DNA, 95 bp, synthetic construct
  misc_feature 1..95: note = Neurod6_1524_RNA
  misc_feature 95: note = RNA
  source 1..95: mol_type = other DNA
tgtgatacagacaagagggactgattcctttgactcacattgcgtctatttagtggagccttgcctatcttctttagagagagagagaatcacag

SEQ ID NO: 188 - DNA, 95 bp, synthetic construct
  misc_feature 1..95: note = Neurod6_168_RNA
  misc_feature 95: note = RNA
  source 1..95: mol_type = other DNA
tctcattgatctctaaaaagctgattcctttgactcacattgcgtctatttagtggagccttgcctatcttctttatctgtgtgtatctgcacta

SEQ ID NO: 189 - DNA, 95 bp, synthetic construct
  misc_feature 1..95: note = Neurod6_1688_RNA
  misc_feature 95: note = RNA
  source 1..95: mol_type = other DNA
agacattgaagtatgctgtgctgattcctttgactcacattgcgtctatttagtggagccttgcctatcttctttcataactgtacaactgaaat

SEQ ID NO: 190 - DNA, 95 bp, synthetic construct
  misc_feature 1..95: note = Neurod6_2041_RNA
  misc_feature 95: note = RNA
  source 1..95: mol_type = other DNA
aacaatacaaaacaagtgctctgattcctttgactcacattgcgtctatttagtggagccttgcctatcttctttacctgtacagaaaaatcctg

SEQ ID NO: 191 - DNA, 95 bp, synthetic construct
  misc_feature 1..95: note = Neurod6_228_RNA
  misc_feature 95: note = RNA
  source 1..95: mol_type = other DNA
ttttcaggctgagtgtcgcactgattcctttgactcacattgcgtctatttagtggagccttgcctatcttctttcattttggatcttccaaatc

SEQ ID NO: 192 - DNA, 95 bp, synthetic construct
  misc_feature 1..95: note = Neurod6_315_RNA
  misc_feature 95: note = RNA
  source 1..95: mol_type = other DNA
gtagtgttaacatggttcttctgattcctttgactcacattgcgtctatttagtggagccttgcctatcttcttttacgacagactcgtcaaacg

SEQ ID NO: 193 - DNA, 95 bp, synthetic construct
  misc_feature 1..95: note = Neurod6_495_RNA
  misc_feature 95: note = RNA
  source 1..95: mol_type = other DNA
tgtcttcttcctcctcttctctgattcctttgactcacattgcgtctatttagtggagccttgcctatcttctttattctcatcttcttcctctc

SEQ ID NO: 194 - DNA, 95 bp, synthetic construct
  misc_feature 1..95: note = Neurod6_648_RNA
  misc_feature 95: note = RNA
  source 1..95: mol_type = other DNA
tgtccagagcatcattgaggctgattcctttgactcacattgcgtctatttagtggagccttgcctatcttctttggggaccacttttcgcaaat

SEQ ID NO: 195 - DNA, 95 bp, synthetic construct
  misc_feature 1..95: note = Neurod6_714_RNA
  misc_feature 95: note = RNA
  source 1..95: mol_type = other DNA
gtcgtaaagtttctattttgctgattcctttgactcacattgcgtctatttagtggagccttgcctatcttctttccagatgtaatttttggcca

SEQ ID NO: 196 - DNA, 95 bp, synthetic construct
  misc_feature 1..95: note = Neurod6_971_RNA
  misc_feature 95: note = RNA
  source 1..95: mol_type = other DNA
cccatgccctgggggagtggctgattcctttgactcacattgcgtctatttagtggagccttgcctatcttctttgacttggaattatcaagagt

SEQ ID NO: 197 - DNA, 92 bp, synthetic construct
  misc_feature 1..92: note = Nov_DO2_ATGC_RNA
  misc_feature 92: note = RNA
  source 1..92: mol_type = other DNA
ggagaaagttcatgacactctacgattttaccagtggctgcgtctatttagtggagccatgcctatcttctttgagtcggtttgtctataat

SEQ ID NO: 198 - DNA, 95 bp, synthetic construct
  misc_feature 1..95: note = Pcp4_120_RNA
  misc_feature 95: note = RNA
  source 1..95: mol_type = other DNA
tcagaaggcaatgctcagggctgattcctttgactcacattgcgtctatttagtggagccatccctatcttctttgctaggtcccacagaacagc

SEQ ID NO: 199 - DNA, 95 bp, synthetic construct
  misc_feature 1..95: note = Pcp4_181_RNA
  misc_feature 95: note = RNA
  source 1..95: mol_type = other DNA
tccggcactttgtctctcacctgattcctttgactcacattgcgtctatttagtggagccatccctatcttctttttgtcttttccgttggtcgc

SEQ ID NO: 200 - DNA, 95 bp, synthetic construct
  misc_feature 1..95: note = Pcp4_305_RNA
  misc_feature 95: note = RNA
  source 1..95: mol_type = other DNA
actgagactgaatggccacactgattcctttgactcacattgcgtctatttagtggagccatccctatcttcttttttcttctggaattttctga

SEQ ID NO: 201 - DNA, 95 bp, synthetic construct
  misc_feature 1..95: note = Pcp4_386_RNA
  misc_feature 95: note = RNA
  source 1..95: mol_type = other DNA
aacttggtgtcttcaggtggctgattcctttgactcacattgcgtctatttagtggagccatccctatcttctttttcttgatggatggtggttg

SEQ ID NO: 202 - DNA, 95 bp, synthetic construct
  misc_feature 1..95: note = Pcp4_472_RNA
  misc_feature 95: note = RNA
  source 1..95: mol_type = other DNA
ttcaggtttgtagcagggtgctgattcctttgactcacattgcgtctatttagtggagccatccctatcttctttatgggtttctcttcatgcat

SEQ ID NO: 203 - DNA, 95 bp, synthetic construct
  misc_feature 1..95: note = Pde1a_1081_RNA
  misc_feature 95: note = RNA
  source 1..95: mol_type = other DNA
ttctctgttgagtccgtcagtctacgagtttgcagtcacgtgcgtctatttagtggagccatcgctatcttctttctataagaggaatgacaatt

SEQ ID NO: 204 - DNA, 95 bp, synthetic construct
  misc_feature 1..95: note = Pde1a_120_RNA
  misc_feature 95: note = RNA
  source 1..95: mol_type = other DNA
actttggtttttcttcaggctctacgagtttgcagtcacgtgcgtctatttagtggagccatcgctatcttctttagcatggacaatgctgcgaa

SEQ ID NO: 205 - DNA, 95 bp, synthetic construct
  misc_feature 1..95: note = Pde1a_1216_RNA
  misc_feature 95: note = RNA
  source 1..95: mol_type = other DNA
tcacacacggagccttttgttctacgagtttgcagtcacgtgcgtctatttagtggagccatcgctatcttctttagtctggggcatagctccca

SEQ ID NO: 206 - DNA, 95 bp, synthetic construct
  misc_feature 1..95: note = Pde1a_273_RNA
  misc_feature 95: note = RNA
  source 1..95: mol_type = other DNA
catttaaggcaaatacatcatctacgagtttgcagtcacgtgcgtctatttagtggagccatcgctatcttctttgctatgctccccgcttgctt

SEQ ID NO: 207 - DNA, 95 bp, synthetic construct
  misc_feature 1..95: note = Pde1a_334_RNA
  misc_feature 95: note = RNA
  source 1..95: mol_type = other DNA
agatcatatctggtaaagagtctacgagtttgcagtcacgtgcgtctatttagtggagccatcgctatcttctttgaatcttgaagcggttgata

SEQ ID NO: 208 - DNA, 95 bp, synthetic construct
  misc_feature 1..95: note = Pde1a_469_RNA
  misc_feature 95: note = RNA
  source 1..95: mol_type = other DNA
atataatgcacagtttgagttctacgagtttgcagtcacgtgcgtctatttagtggagccatcgctatcttcttttgatacctgtatgaagcatt

SEQ ID NO: 209 - DNA, 95 bp, synthetic construct
  misc_feature 1..95: note = Pde1a_615_RNA
  misc_feature 95: note = RNA
  source 1..95: mol_type = other DNA
tgtacagaatagcaacgtcctctacgagtttgcagtcacgtgcgtctatttagtggagccatcgctatcttctttctcaagcactgagcggtcgt

SEQ ID NO: 210 - DNA, 95 bp, synthetic construct
  misc_feature 1..95: note = Pde1a_759_RNA
  misc_feature 95: note = RNA
  source 1..95: mol_type = other DNA
ctgtcgctaagaccatttcatctacgagtttgcagtcacgtgcgtctatttagtggagccatcgctatcttctttctgaaaatgccctgacatgt

SEQ ID NO: 211 - DNA, 95 bp, synthetic construct
  misc_feature 1..95: note = Pde1a_904_RNA
  misc_feature 95: note = RNA
  source 1..95: mol_type = other DNA
ctgtagtgcaacttccaagttctacgagtttgcagtcacgtgcgtctatttagtggagccatcgctatcttctttccattagggccatggtccat

SEQ ID NO: 212 - DNA, 95 bp, synthetic construct
  misc_feature 1..95: note = Pde1a_995_RNA
  misc_feature 95: note = RNA
  source 1..95: mol_type = other DNA
cttccgatcacaaagtggagtctacgagtttgcagtcacgtgcgtctatttagtggagccatcgctatcttctttgactgggcaaccattgttga

SEQ ID NO: 213 - DNA, 95 bp, synthetic construct
  misc_feature 1..95: note = Penk_1282_RNA
  misc_feature 95: note = RNA
  source 1..95: mol_type = other DNA
caatactgagcttcaagacttctacgattttaccagtggctgcgtctatttagtggagccgtacctatcttctttacaacatagccataagagac

SEQ ID NO: 214 - DNA, 95 bp, synthetic construct
  misc_feature 1..95: note = Penk_286_RNA
  misc_feature 95: note = RNA
  source 1..95: mol_type = other DNA
catgggctgtaggagagaagtctacgattttaccagtggctgcgtctatttagtggagccgtacctatcttctttcaaagcctcaggaaccgcgc

SEQ ID NO: 215 - DNA, 95 bp, synthetic construct
  misc_feature 1..95: note = Penk_638_RNA
  misc_feature 95: note = RNA
  source 1..95: mol_type = other DNA
gatatagctcgtccatcttctctacgattttaccagtggctgcgtctatttagtggagccgtacctatcttctttttcttcttctggctccatgg

SEQ ID NO: 216 - DNA, 95 bp, synthetic construct
  misc_feature 1..95: note = Penk_83_RNA
  misc_feature 95: note = RNA
  source 1..95: mol_type = other DNA
tgcctgggactattctatcttctacgattttaccagtggctgcgtctatttagtggagccgtacctatcttctttgtttcctgctgttctagtga

SEQ ID NO: 217 - DNA, 95 bp, synthetic construct
  misc_feature 1..95: note = Penk_882_RNA
  misc_feature 95: note = RNA
  source 1..95: mol_type = other DNA
agttgggggcttcttttgagtctacgattttaccagtggctgcgtctatttagtggagccgtacctatcttctttgctcttttgcttcatcttcc

SEQ ID NO: 218 - DNA, 89 bp, synthetic construct
  misc_feature 1..89: note = Plcxd2_DO3_GAAA_RNA
  misc_feature 89: note = RNA
  source 1..89: mol_type = other DNA
gcactcctacacaatgactgattcctttgactcacattgcgtctatttagtggagccgaaactatcttctttgaagatggtgagggtat

SEQ ID NO: 219 - DNA, 90 bp, synthetic construct
  misc_feature 1..90: note = Plcxd2_DO3_GGCC_RNA
  misc_feature 90: note = RNA
  source 1..90: mol_type = other DNA
gtggtagaaaatgagaacctgattcctttgactcacattgcgtctatttagtggagccggccctatcttcttttgcttgtagaagggaca

SEQ ID NO: 220 - DNA, 95 bp, synthetic construct
  misc_feature 1..95: note = Rorb_2282_RNA
  misc_feature 95: note = RNA
  source 1..95: mol_type = other DNA
tcattcagaattggattccactgattcctttgactcacattgcgtctatttagtggagccaaatctatcttctttataaccaccaaagtgaagtt

SEQ ID NO: 221 - DNA, 95 bp, synthetic construct
  misc_feature 1..95: note = Rorb_4479_RNA
  misc_feature 95: note = RNA
  source 1..95: mol_type = other DNA
tcaattttctgccttaagccctgattcctttgactcacattgcgtctatttagtggagccaaatctatcttctttaagaagaaaaagaagttcat

SEQ ID NO: 222 - DNA, 95 bp, synthetic construct
  misc_feature 1..95: note = Rorb_536_RNA
  misc_feature 95: note = RNA
  source 1..95: mol_type = other DNA
atgtgaggtcatagataggtctgattcctttgactcacattgcgtctatttagtggagccaaatctatcttctttggtaaacaagttgggtacag

SEQ ID NO: 223 - DNA, 95 bp, synthetic construct
  misc_feature 1..95: note = Rorb_6395_RNA
  misc_feature 95: note = RNA
  source 1..95: mol_type = other DNA
gagaaagtgtcacagatttgctgattcctttgactcacattgcgtctatttagtggagccaaatctatcttctttaggtacaattaagagaaagg

SEQ ID NO: 224 - DNA, 95 bp, synthetic construct
  misc_feature 1..95: note = Rorb_8435_RNA
  misc_feature 95: note = RNA
  source 1..95: mol_type = other DNA
tagttgttagggagtgctgcctgattcctttgactcacattgcgtctatttagtggagccaaatctatcttctttaagtaatagaaaactctttt

SEQ ID NO: 225 - DNA, 98 bp, synthetic construct
  misc_feature 1..98: note = Rorb_DO3_CCGG_RNA
  misc_feature 98: note = RNA
  source 1..98: mol_type = other DNA
agccttttaaagtcatatttggtctgattcctttgactcacattgcgtctatttagtggagccccggctatcttcttaatcggtcatcataaaatact

SEQ ID NO: 226 - DNA, 87 bp, synthetic construct
  misc_feature 1..87: note = Rprm_654_RNA
  misc_feature 87: note = RNA
  source 1..87: mol_type = other DNA
cggtccgtgatggtgcgtgcttgtggtagcaaatatgcgtctatttagtggagccttgtctatcttctttgacaggtttgcgttgct

SEQ ID NO: 227 - DNA, 74 bp, synthetic construct
  misc_feature 1..74: note = Sst_432_AP1SWPLP_RNA
  misc_feature 74: note = RNA
  source 1..74: mol_type = other DNA
taacaggatgtgaatgtcttctacgattttaccagtggcctgactatcttcttttaggacaacaatattaaagc

SEQ ID NO: 228 - DNA, 95 bp, synthetic construct
  misc_feature 1..95: note = Synpr_1071_RNA
  misc_feature 95: note = RNA
  source 1..95: mol_type = other DNA
catactagagactttaagcttctacgattttaccagtggctgcgtctatttagtggagccattactatcttctttaaggtaatctatgcacatta

SEQ ID NO: 229 - DNA, 95 bp, synthetic construct
  misc_feature 1..95: note = Synpr_1643_RNA
  misc_feature 95: note = RNA
  source 1..95: mol_type = other DNA
cctctctggatgcaaagaaatctacgattttaccagtggctgcgtctatttagtggagccattactatcttctttaactatggtgtctaaatctg

SEQ ID NO: 230 - DNA, 95 bp, synthetic construct
  misc_feature 1..95: note = Synpr_260_RNA
  misc_feature 95: note = RNA
  source 1..95: mol_type = other DNA
atgtacacgaccgtggcagctctacgattttaccagtggctgcgtctatttagtggagccattactatcttctttggtacttgttctggaagaaa

SEQ ID NO: 231 - DNA, 95 bp, synthetic construct
  misc_feature 1..95: note = Synpr_591_RNA
  misc_feature 95: note = RNA
  source 1..95: mol_type = other DNA
aaggtatctctgtccagaggtctacgattttaccagtggctgcgtctatttagtggagccattactatcttcttttgcttctccatggggtctga

SEQ ID NO: 232 - DNA, 98 bp, synthetic construct
  misc_feature 1..98: note = Synpr_DO2_ATTA_RNA
  misc_feature 98: note = RNA
  source 1..98: mol_type = other DNA
cttaaaaattcttctgctactggtctacgattttaccagtggctgcgtctatttagtggagccattactatcttcttcattaataattgattgaaact

SEQ ID NO: 233 - DNA, 95 bp, synthetic construct
  misc_feature 1..95: note = Yjefn3_138_RNA
  misc_feature 95: note = RNA
  source 1..95: mol_type = other DNA
cactagcgtgcccacatagtcgtgcttgtggtagcaaatatgcgtctatttagtggagcctttactatcttctttggccttggtcacagccaccg

SEQ ID NO: 234 - DNA, 95 bp, synthetic construct
  misc_feature 1..95: note = Yjefn3_344_RNA
  misc_feature 95: note = RNA
  source 1..95: mol_type = other DNA
cttctcgcactgcgtggtcacgtgcttgtggtagcaaatatgcgtctatttagtggagcctttactatcttctttgacaggaaggggatgtccat

SEQ ID NO: 235 - DNA, 95 bp, synthetic construct
  misc_feature 1..95: note = Yjefn3_686_RNA
  misc_feature 95: note = RNA
  source 1..95: mol_type = other DNA
aaactttcggcggacgtcatcgtgcttgtggtagcaaatatgcgtctatttagtggagcctttactatcttcttttattttggcaggtgcaggcc

SEQ ID NO: 236 - DNA, 95 bp, synthetic construct
  misc_feature 1..95: note = Bgn_412_RNA
  misc_feature 95: note = RNA
  source 1..95: mol_type = other DNA
gggcacagtcttcagacccatctacgattttaccagtggctgcgtctatttagtggagccctatctatcttctttgtgtcaggtgagatctcctt

SEQ ID NO: 237 - DNA, 95 bp, synthetic construct
  misc_feature 1..95: note = Bgn_851_RNA
  misc_feature 95: note = RNA
  source 1..95: mol_type = other DNA
tcagggtctcagggagatcttctacgattttaccagtggctgcgtctatttagtggagccctatctatcttctttgtggtccaggtgaagttcgt

SEQ ID NO: 238 - DNA, 95 bp, synthetic construct
  misc_feature 1..95: note = Bgn_1194_RNA
  misc_feature 95: note = RNA
  source 1..95: mol_type = other DNA
tcccagtagggcacagggtttctacgattttaccagtggctgcgtctatttagtggagccctatctatcttctttggaaggtggcaggctgcact

SEQ ID NO: 239 - DNA, 95 bp, synthetic construct
  misc_feature 1..95: note = Bgn_1577_RNA
  misc_feature 95: note = RNA
  source 1..95: mol_type = other DNA
aacaatggcggtggcagtgttctacgattttaccagtggctgcgtctatttagtggagccctatctatcttctttaggaacacatgcctggatgg

SEQ ID NO: 240 - DNA, 95 bp, synthetic construct
  misc_feature 1..95: note = Bgn_2309_RNA
  misc_feature 95: note = RNA
  source 1..95: mol_type = other DNA
tcagggacccaggggtgaggtctacgattttaccagtggctgcgtctatttagtggagccctatctatcttctttgaccatcacctcctaccaca

SEQ ID NO: 241 - DNA, 95 bp, synthetic construct
  misc_feature 1..95: note = Apq4_879_RNA
  misc_feature 95: note = RNA
  source 1..95: mol_type = other DNA
cttaaggcgacgtttgagctctgattcctttgactcacattgcgtctatttagtggagcccattctatcttctttgcggctttgctgaaggcttc

SEQ ID NO: 242 - DNA, 95 bp, synthetic construct
  misc_feature 1..95: note = Apq4_2186_RNA
  misc_feature 95: note = RNA
  source 1..95: mol_type = other DNA
aattacactcacaatgccgactgattcctttgactcacattgcgtctatttagtggagcccattctatcttcttttaattcacacaaatgggtat

SEQ ID NO: 243 - DNA, 95 bp, synthetic construct
  misc_feature 1..95: note = Apq4_3100_RNA
  misc_feature 95: note = RNA
  source 1..95: mol_type = other DNA
cactggaaatgactgttaaactgattcctttgactcacattgcgtctatttagtggagcccattctatcttcttttgtaccatactgaatgctgt

SEQ ID NO: 244 - DNA, 95 bp, synthetic construct
  misc_feature 1..95: note = Apq4_3673_RNA
  misc_feature 95: note = RNA
  source 1..95: mol_type = other DNA
cggtgtatctgtcagtagctctgattcctttgactcacattgcgtctatttagtggagcccattctatcttcttttttcctctctgatctctgtg

SEQ ID NO: 245 - DNA, 95 bp, synthetic construct
  misc_feature 1..95: note = Apq4_4344_RNA
  misc_feature 95: note = RNA
  source 1..95: mol_type = other DNA
acagaggcagtgtctctgtgctgattcctttgactcacattgcgtctatttagtggagcccattctatcttctttgctctctggcttcaattgtc

SEQ ID NO: 246 - DNA, 95 bp, synthetic construct
  misc_feature 1..95: note = Pdgfra_296_RNA
  misc_feature 95: note = RNA
  source 1..95: mol_type = other DNA
tgggaggatagagggtaatatctacgagtttgcagtcacgtgcgtctatttagtggagcctgtcctatcttctttacaatcttctcattctcgtt

SEQ ID NO: 247 - DNA, 95 bp, synthetic construct
  misc_feature 1..95: note = Pdgfra_646_RNA
  misc_feature 95: note = RNA
  source 1..95: mol_type = other DNA
ggtatgatggcagagtcatctctacgagtttgcagtcacgtgcgtctatttagtggagcctgtcctatcttctttccggatctgtggtgcggcaa

SEQ ID NO: 248 - DNA, 95 bp, synthetic construct
  misc_feature 1..95: note = Pdgfra_832_RNA
  misc_feature 95: note = RNA
  source 1..95: mol_type = other DNA
gttgctttcaaggcataaactctacgagtttgcagtcacgtgcgtctatttagtggagcctgtcctatcttcttttctccagattcagttctgac

SEQ ID NO: 249 - DNA, 95 bp, synthetic construct
  misc_feature 1..95: note = Pdgfra_1227_RNA
  misc_feature 95: note = RNA
  source 1..95: mol_type = other DNA
ggtaggcctgcacctccacctctacgagtttgcagtcacgtgcgtctatttagtggagcctgtcctatcttctttccacgatatcctgggcgtcg

SEQ ID NO: 250 - DNA, 95 bp, synthetic construct
  misc_feature 1..95: note = Pdgfra_1544_RNA
  misc_feature 95: note = RNA
  source 1..95: mol_type = other DNA
catccagtcgatttctggaatctacgagtttgcagtcacgtgcgtctatttagtggagcctgtcctatcttctttttcttaatatgcttgcagat

SEQ ID NO: 251 - DNA, 57 bp, synthetic construct
  misc_feature 1..57: note = fwd_index1
  source 1..57: mol_type = other DNA
aatgatacggcgaccaccgagatctacacaggctataacactctttccctacacgac

SEQ ID NO: 252 - DNA, 57 bp, synthetic construct
  misc_feature 1..57: note = fwd_index2
  source 1..57: mol_type = other DNA
aatgatacggcgaccaccgagatctacacgcctctatacactctttccctacacgac

SEQ ID NO: 253 - DNA, 57 bp, synthetic construct
  misc_feature 1..57: note = fwd_index3
  source 1..57: mol_type = other DNA
aatgatacggcgaccaccgagatctacacaggataggacactctttccctacacgac

SEQ ID NO: 254 - DNA, 57 bp, synthetic construct
  misc_feature 1..57: note = fwd_index4
  source 1..57: mol_type = other DNA
aatgatacggcgaccaccgagatctacactcagagccacactctttccctacacgac

SEQ ID NO: 255 - DNA, 57 bp, synthetic construct
  misc_feature 1..57: note = fwd_index5
  source 1..57: mol_type = other DNA
aatgatacggcgaccaccgagatctacaccttcgcctacactctttccctacacgac

SEQ ID NO: 256 - DNA, 57 bp, synthetic construct
  misc_feature 1..57: note = fwd_index6
  source 1..57: mol_type = other DNA
aatgatacggcgaccaccgagatctacactaagattaacactctttccctacacgac

SEQ ID NO: 257 - DNA, 57 bp, synthetic construct
  misc_feature 1..57: note = fwd_index7
  source 1..57: mol_type = other DNA
aatgatacggcgaccaccgagatctacacacgtcctgacactctttccctacacgac

SEQ ID NO: 258 - DNA, 57 bp, synthetic construct
  misc_feature 1..57: note = fwd_index8
  source 1..57: mol_type = other DNA
aatgatacggcgaccaccgagatctacacgtcagtacacactctttccctacacgac

SEQ ID NO: 259 - DNA, 53 bp, synthetic construct
  misc_feature 1..53: note = rev_index1
  source 1..53: mol_type = other DNA
caagcagaagacggcatacgagatcgagtaatgtgactggagttcagacgtgt

SEQ ID NO: 260 - DNA, 53 bp, synthetic construct
  misc_feature 1..53: note = rev_index2
  source 1..53: mol_type = other DNA
caagcagaagacggcatacgagattctccggagtgactggagttcagacgtgt

SEQ ID NO: 261 - DNA, 53 bp, synthetic construct
  misc_feature 1..53: note = rev_index3
  source 1..53: mol_type = other DNA
caagcagaagacggcatacgagataatgagcggtgactggagttcagacgtgt

SEQ ID NO: 262 - DNA, 20 bp, synthetic construct
  misc_feature 1..20: note = P5primer
  source 1..20: mol_type = other DNA
aatgatacggcgaccaccga

SEQ ID NO: 263 - DNA, 21 bp, synthetic construct
  misc_feature 1..21: note = P7primer
  source 1..21: mol_type = other DNA
caagcagaagacggcatacga

SEQ ID NO: 264 - DNA, 77 bp, synthetic construct; identical to SEQ ID NO: 86
  misc_feature 1..77: note = R_KRAS.D3
  misc_feature 24: note = RNA
  misc_feature 40: note = RNA
  misc_feature 56: note = RNA
  source 1..77: mol_type = other DNA

SEQ ID NO: 265 - DNA, 77 bp, synthetic construct; identical to SEQ ID NO: 86
  misc_feature 1..77: note = R_KRAS.D8
  misc_feature 18: note = RNA
  misc_feature 24: note = RNA
  misc_feature 30: note = RNA
  misc_feature 36: note = RNA
  misc_feature 42: note = RNA
  misc_feature 49: note = RNA
  misc_feature 56: note = RNA
  misc_feature 62: note = RNA
  source 1..77: mol_type = other DNA

SEQ ID NO: 266 - protein, 575 aa, Bacteriophage phi-29 [sequence omitted]

SEQ ID NO: 267 - DNA, 77 bp, synthetic construct; identical to SEQ ID NO: 124
  misc_feature 1..77: note = R_KRAS.2G
  misc_feature 40..41: note = RNA
  source 1..77: mol_type = other DNA

SEQ ID NO: 268 - DNA, 77 bp, synthetic construct; identical to SEQ ID NO: 125
  misc_feature 1..77: note = R_KRAS.2C
  misc_feature 40..41: note = RNA
  source 1..77: mol_type = other DNA

SEQ ID NO: 269 - DNA, 77 bp, synthetic construct; identical to SEQ ID NO: 122
  misc_feature 1..77: note = R_KRAS.2A
  misc_feature 40..41: note = RNA
  source 1..77: mol_type = other DNA

SEQ ID NO: 270 - DNA, 77 bp, synthetic construct; identical to SEQ ID NO: 127
  misc_feature 1..77: note = R_KRAS.2U
  misc_feature 40..41: note = RNA
  source 1..77: mol_type = other DNA

SEQ ID NO: 271 - DNA, 77 bp, synthetic construct; identical to SEQ ID NO: 131
  misc_feature 1..77: note = R_KRAS.3G
  misc_feature 40..42: note = RNA
  source 1..77: mol_type = other DNA

SEQ ID NO: 272 - DNA, 77 bp, synthetic construct; identical to SEQ ID NO: 125
  misc_feature 1..77: note = R_KRAS.3C
  misc_feature 40..42: note = RNA
  source 1..77: mol_type = other DNA

SEQ ID NO: 273 - DNA, 77 bp, synthetic construct; identical to SEQ ID NO: 133
  misc_feature 1..77: note = R_KRAS.3A
  misc_feature 40..42: note = RNA
  source 1..77: mol_type = other DNA

SEQ ID NO: 274 - DNA, 78 bp, synthetic construct; identical to SEQ ID NO: 134
  misc_feature 1..78: note = R_KRAS.3U
  misc_feature 40..42: note = RNA
  source 1..78: mol_type = other DNA

SEQ ID NO: 275 - DNA, 77 bp, synthetic construct; identical to SEQ ID NO: 86
  misc_feature 1..77: note = R_KRAS.3
  misc_feature 40..42: note = RNA
  source 1..77: mol_type = other DNA

SEQ ID NO: 276 - DNA, 77 bp, synthetic construct; identical to SEQ ID NO: 86
  misc_feature 1..77: note = R_KRAS.2
  misc_feature 40..41: note = RNA
  source 1..77: mol_type = other DNA

SEQ ID NO: 277 - DNA, 57 bp, synthetic construct; identical to SEQ ID NO: 107
  misc_feature 1..57: note = R_KRAS wt1_2
  misc_feature 20..21: note = RNA
  source 1..57: mol_type = other DNA

SEQ ID NO: 278 - DNA, 57 bp, synthetic construct; identical to SEQ ID NO: 107
  misc_feature 1..57: note = R_KRAS wt1_3
  misc_feature 20..22: note = RNA
  source 1..57: mol_type = other DNA

SEQ ID NO: 279 - DNA, 57 bp, synthetic construct; identical to SEQ ID NO: 107
  misc_feature 1..57: note = R_KRAS wt1_4
  misc_feature 20..23: note = RNA
  source 1..57: mol_type = other DNA

SEQ ID NO: 280 - DNA, 57 bp, synthetic construct; identical to SEQ ID NO: 107
  misc_feature 1..57: note = R_KRAS wt1_5
  misc_feature 20..24: note = RNA
  source 1..57: mol_type = other DNA

SEQ ID NO: 281 - DNA, 57 bp, synthetic construct; identical to SEQ ID NO: 107
  misc_feature 1..57: note = R_KRAS wt1_7
  misc_feature 20..26: note = RNA
  source 1..57: mol_type = other DNA